European Patent Application EP 4 603 574 A1, published August 20, 2025. Title: 파라코커스 아미노보란스 BM109 균주 및 이의 용도. Applicant: 주식회사 바이오미. The sequence listing filed with the application follows.

SEQUENCE LISTING (11 sequences)

SEQ ID NO: 1 - DNA, 1344 bp, Paracoccus aminovorans BM109
  source 1..1344: mol_type = genomic DNA
atgacaaagcgagtcgccgtcatcggcgctggcccttccgggcttgcccagttacgggccttccaatccgccgcccgcaagggcgccgaaatccccgagatcgtctgcttcgagaaacagtcgaactggggcgggctgtggaactacacctggcgcaccggcaccgacgagcacggcgagccggtgcatggctcgatgtatcgctatctctggaccaacggccccaaggaggggctcgagttcgccgactattccttcgaggagcatttcggcaagcagatcgcctcctatccgccgcgcgccgtgatgttcgactatatcgagggccgcgtgctgaaggccggggtccgcgactggatccgcttcaactcggtcatccgctgggtggaattcgacgcggacgccaacgacttcaccgtcaccgtgcacgacatgaaaaaggatcatgtctacaaggagcggttcgaccacgtcatcgtcgcctcggggcatttctcgtcgccgaacgtgccggaatatccgggcttcgaccagttctacggccgcatcacccatgcccacgacttccgcgacgcccgcgagttcgagggccaggacgtgctcatcgtcggctccagctattcggccgaggacatcggctcgcaatgctggaaatacggcgcgaaatcggtgacttcctgctatcgctcggcgccgatgggcttcaaatggcccgacaactgggaagaaaagccggccatggtgcgggtcgaaggcaagaccgtgttcttcagcgacgggtcgagccgcacgatcgacgccatcatcctctgcaccggatacaagcactatttcccgttcctgccggacgatctgcggctgaagacggcgaaccggctggcgacggcggacctctacaagggcgtggtctatgcccacaacccgcgcatgttctatgtcggcatgcaggaccagtggttcaccttcaacatgttcgacgcccaggcctggtatgtgcgcgacatcatcatgggccgcatcgaggtgccgcaggacaagcaggtgctgctggctgacgtggccgagcgcgaggcccgcgaggaagccagcgacgacgtgaaatacgcgatcaagtatcagggcgactatgtgaaggagctgatcgccgagaccgactatcccagcttcgacgtcgatggcgcctgcgcggccttctatgaatggaagcatcacaaggccgtcgacatcatggccttccgcaaccactgctatcgctcggtcatcaccggcaccatggcgccggtgcaccatacgccctggaaagacgcgctggacgactcgatggaagtctatctccagaactga

SEQ ID NO: 2 - DNA, 2676 bp, Paracoccus aminovorans BM109
  source 1..2676: mol_type = genomic DNA
atgactgttttccaacccacgcgacgggcgttcctacggggtggcgttgcagcgatcggtgcggtaggtcttttcggaaccagagcacttgcctcgatcgacccgaactcgttcccggaccggacttttcacgccacccattacggcccgttcaatgccgtggtgaaggacggcaagctcatcggggtgaacgccattcccgagctcgacggtcaacccaacgagatgctgcttttcggtgtggcggaccgcacctatgacgcctcacgcatcgaatatccgatggtccgcaaatcctatctggacaactggcagaccggcgacatcaagcccgaattgcgcggcaaggagccctatgtccgcgtggactgggacaccgcttacagcctgatggccaaggcactgctggacaccgcgtccgaatacggcaaccaggcgatttttagctcctcttatggcggctgggccaacgccggcaacttccgcccgaacgtgatgcaggggcggttcctcaacctgatcgggggctgcacgatcactcagggcgactggtcggccggcgcctcgcagatctgcctgccgcgcgtgatcggcgacatggaggtctactccgcacagactgcttgggaggtgatccgcgacaataccgaggtcttcgtgctggtcggctgcgacccgatcaagaacaaccgcatcgaatacaccgtggccgaccaccagatctatgcaccctggggcgagatccgcgacaacggctgccgtttcatctcgatcaacccgcaacgcacggcgtcggacgactatctggacgccgaatggatcagcatcgtgcccaataccgatgtcgccctgttcagcgccatggcgttccacgtcttggaaaagggcctggaagacaaggaatatatgaaccaatacacggtcggggccgacaagtggatcgcctatatcaagggcaataccgatggcgtgccgaagacgccggaatgggctgccgccatcactgagatcgacgcgagcaagatccgcgaactggccgagctgctggccggatcgaaaacccagatcgccggtgcctggtcgctgcaacgtgcccagcatggcgaaatgacccattgggccatcgtgaactttgccgcgctgaccggcaagatcggcaagcctggccaaggcgtagggttttcctggcattacggcggcggcgggatgccgcaatcgggcaagtccacccccaccggcttgtcgcagggccgcaactgggtcaagaacatctgcccggccagccgcatcaccgagatgctggagcacccgggcgagaaatttacctacaacggcaacgaaggcacctatccagacatcaagatcgtcttcaacgccggcaacaactttatgagccaccagcaggacaccaaccggctgatccgcgccctgaccaaggtcgagcacgtctttagcgtcgacgtatggtggaccgccgcgacccgttgggccgatattgtgctgccggctgcctcgacgctggaacgcgacgacataagcgtcggcggcacctattccaacgacaaggtctttgccatgaagcaggtgatcgagccggtgggcgaaagccgctcggactatcacatcttcgaaggtctggccgacaagatgggcatctggcagcagttcaccgacggactggagctgatcgaccacattcaggccgcctatgagaggtcggccgctgccaagggcacgccgttcgaagagttctgggccaagggctatgcccgccaacccgcccctgtcgaggcccggcgctggacccgccacggcgatttctacaaagatccggccgccaatcctctgcataccgcatctggcaagattgagatgtattgcgaggaaatcgccggcttcaacctggacgactgccccggctatccgatctggatggaaaagcacgagtatctgggtaacgccgaggaggatcaggtccacgtcgtcagcccgcatccgtggtatcggctgcacagccagatggaccagtctgcccgcctgcgcgatctctacaagatccagggacgcgagcctgtgcggatcaaccgtcaggatgccgaaaagcgcggaatcgccgatggcgatctggtcgagatgttcaacgaccgcggcagcatcatcgtgggtgcggtcctgtccgacgacatccggccgggcgtggtatcggtctatgaaggctgctggccttcgctcgacagcaaggggcgatgcaactccggcctggtgaactttctgacctcgacacagaggtcttcgggcttgtcgcaggcaacgactgcaaacaccgttctgtgccggatgcgcaagtgcgaggacgccgaagggccgaaccgcgcctatgaaaagccagagatcatcgaggattacgaggtcgccgccatcgacgaggaggttctcggtcttgaccgtgtcgcaacgatcatggaagcgctgctcgcagacgcgaccgagggtgaaaaaatcttctatgagcgctgcacggtatgccatggaccccgtgaagtgtcccactttacccagaaccaatggaaggggatcaccccatccatgttcccccgcgctggtctggacgagaacgaggcggcgctggtcacgcaattcctgatggaaaacgcttcggacgcgccgaagaaatga

SEQ ID NO: 3 - DNA, 2199 bp, Paracoccus aminovorans BM109
  source 1..2199: mol_type = genomic DNA
atgactaacgccagaccggccaaatacgacatcctgttcgagccgatccagctcggtcccaagaccatgaagaaccgctttcaccaaagcccgcactgcatcggcgccggcaccgaccggcccggtttccagatggcgcaccgcggcgtgaaggcggaaggcggctggggcgcgatcaataccgagtattgctcgatccacccggaatccgacgacaccatgcgagtttccgcccggatctgggacgcgggcgacgtgcgcaacctgcgcgccatgtgcgacgaggtgcacaaatacggcgcccttgccggcatcgagatgtggtacggcggcggtcacgccccgaacatggaatcgcgccagacgccgcgcggccccagccagtatgcgtcggaattcgaaacgctgacctattgcaaggagatggacgaggacgacatccggcaggtgcagcagttctacgtggacgccgcgctgcgggcccgcgatgcgggtttcgacatcgtcaacgtctatggcggccacgcctatggcccgatgcagtggctgagcccctatttcaacaagcgcaccgacggctacggcggctcggtcgagaaccgcgcccgtttctggatcgagacgctggaaaaggtcaggagggcggtcggcgacgattgcgccatcgcctcgcgctgcgccatcgacacgctctacggccccggcgggcttgaggtcgaggtggacggcgtgcgcctgatcgagatggccgacgacctggtcgacgtctgggacatcaacgtcggcgacatcgcccaatggggcgaggacgcggcgccgtcgcgcttccagcgtcagggccacgcgatcccctggcagcgcttcgtcaagatgcactcgaaaaagcccgtgctgggcatcggccgcttcaccgatcccgagaagatggccgaggtcatccgcaacggcgaactggacatcatcagctgcgcgcggccctcgatcgccgaccccttcctgcccgagaagatcgagcagggccggcttgacgacatccgcacctgcatcggctgcaacgtctgcatctcgcgctgggaaatcggcggcccgccgatgatctgcacccagaacgccaccgccggcgaggaataccgccgcagctggcaccccgagaagttcgagaaggcgaaatccgacgataccgtgctggtggtcggcgccggtccgtccggctcggaggcggcacgggtgctgctggagcgcggctacgtcacccatctcgtagacagcgccgaaaaggtcggcggccacctgaacgacgtcgccaccctgccgggcctgggcgagtggggctttcaccgcgactatcgcgaggtccagctcaacaagctcgtcaagcgggtcaaggggtcgcagctggcgctcggccagaagcggctgacggcggacgacgtgctggactatggcgccgagaaggtcatcatcgccaccggctcgtcctggaacaccgacggcaccaactgcctcagccacgaccccattccgggcgtcgatgccagcaagccgaaccaggtcacgcccgagcagatcttccgcggcgagaagccgatcggcaagcgcgtcgtgatcctgaacgccgacacctatttcatggccccctcgcttgccgaacagctggcggccaagggtcacgaggtgacggtgatcagcggcgtcgacttcggtcattacatgcacttctcgctggaatacccgaacatgcgccgccgcatgatcgagctgaacgtcaacatcatcggcgaagcctgggcatcgcgggtcgaggacgggcggatcgagtattacgacatctgggccgaaggctcgcggcgcgaataccgcggccccggcaagctgccgcgggacgagaacaagagccatcagtggcttgagttcgatacgctggtcctgaccaccgggcgccattccgactcgtcgctgttcaacgagctcaaggcgcggcgcggcgaatgggaagagaagggcatcaaggacgtctatgtgatcggcgacgcctgggcgcccaagctgatcgccgacgccaccttcgacggccaccgcatcgcccgcgagatcgaggacgccgatccgcagcacccgctgccctacaagcgcgaggtcatctcctggggcacggcctatcagcccggcggcgaatacaagctggaatggcggctctga

SEQ ID NO: 4 - DNA, 2208 bp, Paracoccus aminovorans BM109
  source 1..2208: mol_type = genomic DNA
atgaccagggacccaagattcgacattcttttcacgccgctcaagctgggcccgaaaacgatacgaaacaggttctaccaggttccgcattgcaacggcgccggcaccaatgcgcccggcatgaacatggcccatcgcggcgtcaaggccgaaggcggctggggcgcggtcaataccgagcaatgctcgatccaccccgaatgcgacgacacgctgcggatcaccgcccggatctgggaccagggcgacatgcgcaacctgcgcgccatggtcgatcacgtccacagccacggctcgcttgcgggctgcgaactgttctatggcggcccgcatgccccggggctggaatcgcgcaccatctcgcgcgggcccagccaatatgcctcggaattcggcacggtgccgggctgcccgggcttcacctacaaccacgccgccgacaaggacgagttgcaccggcttcagcagcaatatgtcgatgcggcgctgcgggcccgcgacaccggcttcgacctggtcaacgtctatggcgcccatgcctatgggccgatgcaatggctgaacccgttctacaaccgccgcaccgacgaatacggcggcagtttcgagaaccgggcccggttctggatcgagacgctggaaaagatccgccgggccgtcgatgacgacgtcgcgctggtgacgcgctgcgcggtcgatacgctttacggcggcaagggggtcgagctgggcgaggacgggctgaagttcatcgaactggcctcgccctatctggacctgtgggacgtcaatatcggcgacatcgccgaatggggcgaggatgcgggcccgtcgcgcttctaccagatcgcgcatgagaacgactggatccgccacatcaagcaggcgaccaacaagcccgtcgtcggcgtcggccgctattacgaccctgagaagatgctccaggtcgtcaacgccggcatcgtcgacatcatcggcgccgcgcggccctcgatcgccgatccctggctgccgcgcaagatcgacgagggccgcgtggacgacatccgcacctgcatcgggtgcaacgtctgcatctcgcgctgggaaatgggcggggtgccgttcatctgcacccagaacgccaccgcgggcgaggaataccgccgcggctggcaccccgagaagttcgagaaggcgaagtcggaccacgacgtgctgatcgtcggcgccggtcccgccggctcggaatgcgcgcgggtgctgatggagcgtggctatacggtgcatttggtggacaaggccgagaagatcggcggctatgtcaacgacgtcgccacgttgcccggcttggccgaatggagctttcaccgcgactatcgcgagaaccagctgcaaaagctggtcaagaagaacaaggccagccagatcgcccttggcggcaagccgatgacggcggacgacgtgctgacctatggcgcctcgcgggtgatcatcgccaccggcgcgcgctggagcgaaaccggcgtgaactacaagacccatgccccgatcccgggcgcggacgccagcctgccccatgtcctgacccccgaacaggtgttccagggcaaggcggtcggcaagcgggtcatgatcgtcaactacgacccctattacatggcgcccagcctggccgagaaattcgcccgcgccggccatgaggtcaccgtcgccaccacctgcggcctgggcgcctatatggaatacacgctggaaggcgcgaacatgcagcggctgatccacgagctggggatcaacgtgatcggcgagaccggctgttcccggatcgagccgggccgggtcgagctcttcaacctgtggggcgaaggctacaagcgccagttcaacggcaccgggaaactgccgcgccgggaaaacgacagccacggctggcacgaatgcgacagcgtgatcctggtcaccggccgcgtgtcgcaggacggcctgtatcgcgagttgaaggcgcgcaaggacgagtgggagaagaatggcatcgccgaagtcttcgtcatcggcgatgccgaatcgccgcggctgatcgccgacgcgaccttcgacggccaccggctggcgcgcgagatcgaggacgaggacccgcagcaccagaccccttacaagcgcgaacagcgcgcttggggaaccccctatctgccgggcgaaaaccccgatctggaatggcggctctga

SEQ ID NO: 5 - DNA, 1182 bp, Paracoccus aminovorans BM109
  source 1..1182: mol_type = genomic DNA
atgagcaacagaggcgtcgtctacatcggccctggcaaggtcgaggtccagaacatcgcggacccgaagctgcaatcccccgacgggcgcaagatcgagcatggcgtgatcctgaaggtggtctcgaccaacatctgcggctcggaccagcacatggtgcgcggccgcaccaccgccgaaccgggcctggtgctgggccatgagatcaccggcgaggtgatcgagaagggtgccgacgtcgaaatgctggacatcggcgacatcgtctcggtgccgttcaacgtcgcctgcggccgctgccgctgctgccgtgaaggcgataccggcgtctgcctgacggtgaacccttcgcgcgcggggggcgcctatggctatgtcgacatgggcggctggatcggcggccaagcccgctatgtcatggtgccctatgccgatttcaacctgctgaaattcccggaccgcgaccgcgccctgtccaagatccgcgacctgaccatgctgtcggacatcctgcccaccggcttccacggtgcggtcaaggccggcgtcggcgtgggttccgtggtctatgtcgcgggcgccggcccggtgggtctggcggccgccgcctcggcccgcatcctgggcgcggccgtggtgatgatcggcgacttcaacaaggaacgccttgagcacgcccgcaaggtcggcttcgagccggtggacctgtcgaaatccgaccgtctgggcgacatgatcgccgagatcaccggcacgcccgaggttgattcggccatcgacgccgtgggcttcgaggcgcgcggccattccggcggcgaacagccggccatcgtgctgaaccagatgatggagatcacccgcgccgccggccagatcggcatccccgggctttacgtcaccgaggatccgggcgcggtcgacagtgccgccaagcagggcagcctgtcgatgcgcttcggcctgggctgggccaaggcgcagtcgctgcacaccggccagacgccggtgctgaagtacaaccgccagctcatgcaggcgatcctgcacgaccggctgccgatcgccgacatcgtgaacgcgacgatcatcccgctggacgaggccgtcgccggctacgaaagcttcgaccacggcgtcgccaagaagttcgtgctggatccgcatggcagcctggcggcctga

SEQ ID NO: 6 - DNA, 1203 bp, Paracoccus aminovorans BM109
  source 1..1203: mol_type = genomic DNA
atggccaaggtagtttgcgttctctacgacgatccggtcgacggctatccgacctcttatgcccgcgattccctgccggtgatcgagcgctatcccgacgggcagaccctgcccacgcccaaggccatcgacttcgtgccgggcagcctgctcggttcggtctcgggcgagctgggcctgcgcaactacctggaagcgcagggccacgaactggtggtgacctcgtccaaggacggccccgacagcgagctggaaaagcacctgcacgatgccgaggtggtcatctcgcagccgttctggccggcctacctgaccgccgagcgcatcgccaaggcgccgaagctgaagctggcgctgaccgccggcatcggctcggaccatgtcgacctgcaagccgccatcgaccgcggcatcaccgtggccgaggtgaccttctgcaactcgatcagcgtgtcggaacatgtggtgatgacggcgctgaacctggtgcggaactataccccctcgcatgaatgggcggtgaagggcggctggaacatcgccgattgcgtcacccgctcctatgacatcgaggggatgcatgtcggcaccgtcgccgccggccgcatcggccttgccgtgctgcgccgcttcaagcccttcggcatgcacctgcactataccgaccgccaccgcctgccgcgcgaggtcgaattggagctggacctgacctggcacgagagccccaaggacatgtatccggcctgcgacatcgtcacgctgaactgcccgctgcaccccgagaccgagcatatggtcaacgacgagacgctgaagctgttcaagcgcggcgcctatctggtcaacacggcgcgcggcaagctgtgcgaccgcgacgcggtggcccgggcgctggaaagcggccagctggccggctatggcggcgatgtctggttcccgcagccggcgccgcaggatcatccctggcgcaccatgccgcataacgcgatgacgccgcatatctcgggcacctcgctttcggcgcaggcgcgttatgcggccggcacgcgcgagatcctggaatgctatttcgagggccggccgatccgcgacgaatacctgatcgtgcagggcggcagcctggccggcgtcggcgcgcattcctattccaagggcaatgcgaccggcggctcggaagaggcggcgaagttcgagaaggtctga

SEQ ID NO: 7 - DNA, 600 bp, Paracoccus aminovorans BM109
  source 1..600: mol_type = genomic DNA
atgaacatcgacctctcgcggcgcggcttcctgaagctggcgggtgcgggtgtcgcggcaacgtcgctgggggccatgggcttcggcgaggccgaggcggcagagcaggcgcatgtgcgcgccttcaagctggcctcgatgaccgagacccggaacacctgcacctattgctcggtcgcctgcggcatcctgatctattccaagggcgacgtggccgccggcgaacaggccgagatcatccatatcgaaggcgacgccgaccacccgaccaaccgcggcacgctgtgcccgaaaggcgcggcgctgaaggacatcgtccattccgagacccgcctgaccacgccgcgcatccgccgccccggcaccgacaccttccaggacatcggctgggacgaggcgctggacaagatcgcccgcgcgctgaaggacgaccgcgacgccaacatggtgctgaccaacgacgatggcgtgccggtgaaccgctggacgacgaccggcttcctggccgcctcggccaccacgaacgaaaccgcatggctgacctacaagacggtgcgcgccatggggatcgtcggattcgacaaccaggcgcgcgtctga

SEQ ID NO: 8 - DNA, 2436 bp, Paracoccus aminovorans BM109
  source 1..2436: mol_type = genomic DNA
atgaccaacccctggaccgacatcaagaacaccgacctggtgatcgtgatgggcgggaatgccgccgaagcccatccctgcggcttcaaatgggtgaccgaagccaaggcgcatcgtggcgccaagctgatcgtcgtggaccctcggttcacgcgcacggcctcggtgtccgactattacgcgccgatccggcccgggtccgacatcaccttcctgatggccatgatcaactggatgatccagaacgataaggtccagtgggaatatgtgaagaacttcaccaatgcgcccttcatcgtgaaggacgagttcggctggagcgacgggctgttctcgggctacgaccccgaaaagcgcgactatgacaagtcgagctgggattacgtcatcggcgacgacggctttgccgccgtggacatgaccctgcagcacccgcgctgcgtctggaacctgctcaaggagcatgtctcgcgctatacgccggaactggtcgagcaggtctgcggcacgcccaaggaccgtttcctgcatatcgcggaaatgatcggcgcatgttcggcgcccgacaagaccatgacctcgatgtatgcgctgggctggacgcagcattccaagggcgcgcagaacatccgcggcatggcgatgctgcaactggtgctgggcaatatcggcgtgcgcggcggcggcatgaacgccttgcgcgggcattccaacatccagggcctgaccgacatcgggctgatgtcgaacctgatcccgggctatctgaacatcccgaccgaaaaggaagcggactgggcgacctatatgtccagccgcgaattcaagccgctgcggccgggccagaccagctattggcagaactatcccaagttcatggtcagcttcatgaaggccatgtggggcgatgccgcgacggtcgaaaacgactgggcctatcactacttgcccaagctggacgtgccgacctacgacatcctgcgcatgttcgagctgatgaaggccggcaagatcaccaactacttctgccagggcttcaacccgcttctggccttcccgaaccgggccaagctgaccgaggcgctgtcgaagctgaagctgctggtcatcatggacccgttggagaccgagaccgcgcgcttctgggaaaaccacggcgaatacaacgaggtggacccggccgcgatccagaccgaggtgatccagctgccgaccacctgctttgccgaggacgacggttcgctggtgaactcggggcgctggctgcaatggcattgggcggcgggcacgcctccgggccagtccaagcgcgacacttggatcatgtcgcagatcttccagcgcgtcaggaagctttaccaggacgaaggcggcatcttccccgacccgatcctgaacctgacctgggattatgccgatcccgaggagccgaccgccgaggaactggcgaaagagatgaacggccgcgccctgaaggacgtctacgacctcaaggacacggccaagctgctgacgccggcgggcaagcagctgctgaacttcagccagtatcgcgacgacggctcgaccatgggcggctgctggatcttctcgggctgctggaacgaggacggcaacatgatggcgcggcgggacaatgccgatcccgacgacaccggcatgttcccgaactggacctatgcctggccgctgaaccggcgcgtgctctacaaccgcgcctcggcagacatgcagggcaagccctgggacccgtcgcgcaagctgatggaatgggacggcgagaaatgggcgggctacgacgtgcccgacatcgcccccacctcgaaacccggcgaggtcggccccttcatcatgaaccaggaggggacatcgcgtctctttacccggggcatgatgcgcgacgggccgttcccgacgcatatggagcccttcgagtcgccgatcgccaacccgttcaacgctgagatgcggggcaatccggtggcgcgggtgttcgtggacgatgccgagcaattcgccaccagcgaggaattcccgcttgtcgcgacctcctatcgcctgaccgaacatttccactactggaccaagaacaaccgcatcaacgccgcgctgcagcccgaattcttcgtcgagatcagcaaggaactcgccgccgaaaagggcatcaccaagggcggcatggtgcgggtctggtccaagcgcggctcgatcaaggcgcgggcgctggtgaccggccggatcaagccgctgcaatgcggcgacaagctggtccatgtcgtcggcatcccgctgcactggggcttcgtcggcgcggcgcgcaaagggttcgggccgaacagcctgacgcccttcgtcggcgacgccaacgtggaaacgcccgaattcaaggcgttcctcgtcaatatcgagccagcgacaggggaggcggtatcatga

SEQ ID NO: 9 - DNA, 984 bp, Paracoccus aminovorans BM109
  source 1..984: mol_type = genomic DNA
atgactcaggacccgaacctcgacagcccgcggacggcggtctcgaacccgccggtgcagccgatgccggccaaccttggcgcgggcgacgtggtccgcgcctcggccatgcccaacctgcccccgcccgagcgtgagctgacgccggtggcgaaactgatcgacgtcagcaaatgcatcggctgcaaggcctgccaatcggcctgcgcggaatggaacgacacccatcccgagatcggccacaacaccggggtctatgaaaaccccgcggacctctcgcccgagatgttcacgctgatgcgcttcagcgaatacgaaaacccccagaccggggatttcgaatggctgatccgcaaggacggctgcatgcattgcgccgatcccggctgcctcaaggcctgcccggccccgggcgccatcgtgcaatattccaacggcatcgtggatttcatccacgagaactgcatcggctgcggctattgcgtcaccggctgccccttcgacatcccgcgcgtcagccaaaagacccatgtcagctacaaatgcacgctgtgctcggaccgggtggcggtgggccaggggccggcctgcgccaaggcctgcccgacccaggccatcgtcttcggcaccaaggaggacatggtcgcccatgccgaggcccgggtcgaggatctgaaatcgcgcggctacgacaacgccggcatctacgacccggcgggggtgggcggtacgcatgtcttttacgtgctgcatcacgccgaccagccggggctttatgccgacctgccggccgatccgcagatctcgccggtggtgcgcggctggaagggcgtgaccaagaccgtgggccttgccgccatcggccttgccgccatcggctcggtgctgcacgggttgctgggccgcgccaacaccgtcagcgccgaggacgagcacgaggccgaggagctggtggatcacacccagggaacggagaaggcgtga

SEQ ID NO: 10 - DNA, 687 bp, Paracoccus aminovorans BM109
  source 1..687: mol_type = genomic DNA
atggcgaaccggctttattcccaacccggcgaccggatcgagaccaccgatccggtgaccgtcaaccgctatcgcggcttcacccgcgccaaccactgggtgacggccgccagcctgatcgtgcttttgctgtcgggcatggcgctgttccatccgtcgctgttcttcctgaccgggatcttcggcggcggccagaccacacgctggctgcaccccttcgtcggcatcctgctgttcttcagcttcctgatcctgttcctgcagctctggcggctgaacctgcccaagcccgaggataccacctgggtcagccacatcggcgaggtggtgaagggcgaagaggaaaagctgcccgaacttggcaagtacaatgccgggcagaagttcatcttctgggcgatgtcggcgctgatcgtggtgctgatcgtcacgggcgtgatgatctgggaacagtatttcccggatctggtcagcatccccgtgcgccgctgggcggtgctggtgcattcgctggcggcggtggcgatcatcctggtcttcatcctgcacgtctatgcggcgttctggacccgcggtacgctgcgcgccatgacccgcggcaccgtcaccggcggctgggcctggaagcatcaccgcaaatggctgcgggaactggctggacgcgaccgccgcggcccggcagagtag

SEQ ID NO: 11 - DNA, 4707 bp, Paracoccus aminovorans BM109
  source 1..4707: mol_type = genomic DNA
atgaacatcgacctctcgcggcgcggcttcctgaagctggcgggtgcgggtgtcgcggcaacgtcgctgggggccatgggcttcggcgaggccgaggcggcagagcaggcgcatgtgcgcgccttcaagctggcctcgatgaccgagacccggaacacctgcacctattgctcggtcgcctgcggcatcctgatctattccaagggcgacgtggccgccggcgaacaggccgagatcatccatatcgaaggcgacgccgaccacccgaccaaccgcggcacgctgtgcccgaaaggcgcggcgctgaaggacatcgtccattccgagacccgcctgaccacgccgcgcatccgccgccccggcaccgacaccttccaggacatcggctgggacgaggcgctggacaagatcgcccgcgcgctgaaggacgaccgcgacgccaacatggtgctgaccaacgacgatggcgtgccggtgaaccgctggacgacgaccggcttcctggccgcctcggccaccacgaacgaaaccgcatggctgacctacaagacggtgcgcgccatggggatcgtcggattcgacaaccaggcgcgcgtctgaatgaccaacccctggaccgacatcaagaacaccgacctggtgatcgtgatgggcgggaatgccgccgaagcccatccctgcggcttcaaatgggtgaccgaagccaaggcgcatcgtggcgccaagctgatcgtcgtggaccctcggttcacgcgcacggcctcggtgtccgactattacgcgccgatccggcccgggtccgacatcaccttcctgatggccatgatcaactggatgatccagaacgataaggtccagtgggaatatgtgaagaacttcaccaatgcgcccttcatcgtgaaggacgagttcggctggagcgacgggctgttctcgggctacgaccccgaaaagcgcgactatgacaagtcgagctgggattacgtcatcggcgacgacggctttgccgccgtggacatgaccctgcagcacccgcgctgcgtctggaacctgctcaaggagcatgtctcgcgctatacgccggaactggtcgagcaggtctgcggcacgcccaaggaccgtttcctgcatatcgcggaaatgatcggcgcatgttcggcgcccgacaagaccatgacctcgatgtatgcgctgggctggacgcagcattccaagggcgcgcagaacatccgcggcatggcgatgctgcaactggtgctgggcaatatcggcgtgcgcggcggcggcatgaacgccttgcgcgggcattccaacatccagggcctgaccgacatcgggctgatgtcgaacctgatcccgggctatctgaacatcccgaccgaaaaggaagcggactgggcgacctatatgtccagccgcgaattcaagccgctgcggccgggccagaccagctattggcagaactatcccaagttcatggtcagcttcatgaaggccatgtggggcgatgccgcgacggtcgaaaacgactgggcctatcactacttgcccaagctggacgtgccgacctacgacatcctgcgcatgttcgagctgatgaaggccggcaagatcaccaactacttctgccagggcttcaacccgcttctggccttcccgaaccgggccaagctgaccgaggcgctgtcgaagctgaagctgctggtcatcatggacccgttggagaccgagaccgcgcgcttctgggaaaaccacggcgaatacaacgaggtggacccggccgcgatccagaccgaggtgatccagctgccgaccacctgctttgccgaggacgacggttcgctggtgaactcggggcgctggctgcaatggcattgggcggcgggcacgcctccgggccagtccaagcgcgacacttggatcatgtcgcagatcttccagcgcgtcaggaagctttaccaggacgaaggcggcatcttccccgacccgatcctgaacctgacctgggattatgccgatcccgaggagccgaccgccgaggaactggcgaaagagatgaacggccgcgccctgaaggacgtctacgacctcaaggacacggccaagctgctgacgccggcgggcaagcagctgctgaacttcagccagtatcgcgacgacggctcgaccatgggcggctgctggatcttctcgggctgctggaacgaggacggcaacatgatggcgcggcgggacaatgccgatcccgacgacaccggcatgttcccgaactggacctatgcctggccgctgaaccggcgcgtgctctacaaccgcgcctcggcagacatgcagggcaagccctgggacccgtcgcgcaagctgatggaatgggacggcgagaaatgggcgggctacgacgtgcccgacatcgcccccacctcgaaacccggcgaggtcggccccttcatcatgaaccaggaggggacatcgcgtctctttacccggggcatgatgcgcgacgggccgttcccgacgcatatggagcccttcgagtcgccgatcgccaacccgttcaacgctgagatgcggggcaatccggtggcgcgggtgttcgtggacgatgccgagcaattcgccaccagcgaggaattcccgcttgtcgcgacctcctatcgcctgaccgaacatttccactactggaccaagaacaaccgcatcaacgccgcgctgcagcccgaattcttcgtcgagatcagcaaggaactcgccgccgaaaagggcatcaccaagggcggcatggtgcgggtctggtccaagcgcggctcgatcaaggcgcgggcgctggtgaccggccggatcaagccgctgcaatgcggcgacaagctggtccatgtcgtcggcatcccgctgcactggggcttcgtcggcgcggcgcgcaaagggttcgggccgaacagcctgacgcccttcgtcggcgacgccaacgtggaaacgcccgaattcaaggcgttcctcgtcaatatcgagccagcgacaggggaggcggtatcatgaatgactcaggacccgaacctcgacagcccgcggacggcggtctcgaacccgccggtgcagccgatgccggccaaccttggcgcgggcgacgtggtccgcgcctcggccatgcccaacctgcccccgcccgagcgtgagctgacgccggtggcgaaactgatcgacgtcagcaaatgcatcggctgcaaggcctgccaatcggcctgcgcggaatggaacgacacccatcccgagatcggccacaacaccggggtctatgaaaaccccgcggacctctcgcccgagatgttcacgctgatgcgcttcagcgaatacgaaaacccccagaccggggatttcgaatggctgatccgcaaggacggctgcatgcattgcgccgatcccggctgcctcaaggcctgcccggccccgggcgccatcgtgcaatattccaacggcatcgtggatttcatccacgagaactgcatcggctgcggctattgcgtcaccggctgccccttcgacatcccgcgcgtcagccaaaagacccatgtcagctacaaatgcacgctgtgctcggaccgggtggcggtgggccaggggccggcctgcgccaaggcctgcccgacccaggccatcgtcttcggcaccaaggaggacatggtcgcccatgccgaggcccgggtcgaggatctgaaatcgcgcggctacgacaacgccggcatctacgacccggcgggggtgggcggtacgcatgtcttttacgtgctgcatcacgccgaccagccggggctttatgccgacctgccggccgatccgcagatctcgccggtggtgcgcggctggaagggcgtgaccaagaccgtgggccttgccgccatcggccttgccgccatcggctcggtgctgcacgggttgctgggccgcgccaacaccgtcagcgccgaggacgagcacgaggccgaggagctggtggatcacacccagggaacggagaaggcgtgaatggcgaaccggctttattcccaacccggcgaccggatcgagaccaccgatccggtgaccgtcaaccgctatcgcggcttcacccgcgccaaccactgggtgacggccgccagcctgatcgtgcttttgctgtcgggcatggcgctgttccatccgtcgctgttcttcctgaccgggatcttcggcggcggccagaccacacgctggctgcaccccttcgtcggcatcctgctgttcttcagcttcctgatcctgttcctgcagctctggcggctgaacctgcccaagcccgaggataccacctgggtcagccacatcggcgaggtggtgaagggcgaagaggaaaagctgcccgaacttggcaagtacaatgccgggcagaagttcatcttctgggcgatgtcggcgctgatcgtggtgctgatcgtcacgggcgtgatgatctgggaacagtatttcccggatctggtcagcatccccgtgcgccgctgggcggtgctggtgcattcgctggcggcggtggcgatcatcctggtcttcatcctgcacgtctatgcggcgttctggacccgcggtacgctgcgcgccatgacccgcggcaccgtcaccggcggctgggcctggaagcatcaccgcaaatggctgcgggaactggctggacgcgaccgccgcggcccggcagagtag